European Patent Application EP 4 467 141 A1, published November 27, 2024. Title: SELECTIVE INHIBITORS OF GENOTOXIC STRESS-INDUCED IKK/NF- κB PATHWAYS FOR CANCER THERAPY. Applicant: Max-Delbrueck-Centrum fuer Molekulare Medizin in der Helmholtz-Gemeinschaft. Application EP. The sequence listing filed with the application follows.

SEQUENCE LISTING (11 sequences)

SEQ ID NO: 1 - DNA, 20 bp, synthetic construct
  source 1..20: mol_type = other DNA
ttcggccgagttgtacaatg

SEQ ID NO: 2 - DNA, 20 bp, synthetic construct
  source 1..20: mol_type = other DNA
agcacgttgatctcaagtcg

SEQ ID NO: 3 - DNA, 22 bp, synthetic construct
  source 1..22: mol_type = other DNA
cgagctcgttcagaaatccaag

SEQ ID NO: 4 - DNA, 22 bp, synthetic construct
  source 1..22: mol_type = other DNA
tagcatctggacacatcggaag

SEQ ID NO: 5 - DNA, 20 bp, synthetic construct
  source 1..20: mol_type = other DNA
ttgggtgctgatgtcaatgc

SEQ ID NO: 6 - DNA, 20 bp, synthetic construct
  source 1..20: mol_type = other DNA
acaccaggtcaggattttgc

SEQ ID NO: 7 - DNA, 20 bp, synthetic construct
  source 1..20: mol_type = other DNA
aattccatggcaccgtcaag

SEQ ID NO: 8 - DNA, 20 bp, synthetic construct
  source 1..20: mol_type = other DNA
atcgccccacttgattttgg

SEQ ID NO: 9 - DNA, 22 bp, synthetic construct
  source 1..22: mol_type = other DNA
tacactgaattcacccccactg

SEQ ID NO: 10 - DNA, 22 bp, synthetic construct
  source 1..22: mol_type = other DNA
tgctgcttacatgtctcgatcc

SEQ ID NO: 11 - RNA, 19 nt, synthetic construct
  source 1..19: mol_type = other RNA
gctgcatcatctttgaata